European Patent Application EP 4 306 644 A1, published January 17, 2024. Title: Mutant of Corynebacterium glutamicum with enhanced L-lysine productivity and method for preparing L-lysine using the same. Applicant: DAESANG CORPORATION. The sequence listing filed with the application follows.

SEQUENCE LISTING (16 sequences)

SEQ ID NO: 1 - DNA, 200 bp, Artificial Sequence
  Promoter sequence of lysA gene
cagtcgaggcggcaagaactgctactaccctttttattgtcgaacggggcattacggctccaaggacgtttgttttctgggtcagttaccccaaaaagcatatacagagaccaatgatttttcattaaaaaggcagggatttgttataagtatgggtcgtattctgtgcgacgggtgtacctcggctagaatttctcccc

SEQ ID NO: 2 - DNA, 200 bp, Artificial Sequence
  Mutant promoter sequence of lysA gene
cagtcgaggcggcaagaactgctactaccctttttattgtcgaacggggcattacggctccaaggacgtttgttttctgggtcagttaccccaaaaagcatatacagagaccaatgatttttcattaaaaaggcagggatttgttataagtatgggtcgtattctgtgcgacgggtgtacctctgctagaatttctcccc

SEQ ID NO: 3 - DNA, 200 bp, Artificial Sequence
  Mutant promoter sequence of lysA gene
cagtcgaggcggcaagaactgctactaccctttttattgtcgaacggggcattacggctccaaggacgtttgttttctgggtcagttaccccaaaaagcatatacagagaccaatgatttttcattaaaaaggcagggatttgttataagtatgggtcgtattctgtgcgacgggtgtacctgagctagaatttctcccc

SEQ ID NO: 4 - DNA, 200 bp, Artificial Sequence
  Mutant promoter sequence of lysA gene
cagtcgaggcggcaagaactgctactaccctttttattgtcgaacggggcattacggctccaaggacgtttgttttctgggtcagttaccccaaaaagcatatacagagaccaatgatttttcattaaaaaggcagggatttgttataagtatgggtcgtattctgtgcgacgggtgtacctgtgctagaatttctcccc

SEQ ID NO: 5 - DNA, 30 bp, Artificial Sequence
  lysA-LA-F1
tgattacgcctccgcgaggctgcactgcaa

SEQ ID NO: 6 - DNA, 20 bp, Artificial Sequence
  lysA-LA-F2
tccgcgaggctgcactgcaa

SEQ ID NO: 7 - DNA, 20 bp, Artificial Sequence
  lysA-LA-R1
gtacacccgtcgcacagaat

SEQ ID NO: 8 - DNA, 20 bp, Artificial Sequence
  lysA-LA-R2
tctagcagaggtacacccgt

SEQ ID NO: 9 - DNA, 30 bp, Artificial Sequence
  lysA-RA-F1
ctctgctagaatttctccccatgacaccag

SEQ ID NO: 10 - DNA, 20 bp, Artificial Sequence
  lysA-RA-F2
atttctccccatgacaccag

SEQ ID NO: 11 - DNA, 20 bp, Artificial Sequence
  lysA-RA-R1
gcacacgacccaaagagtca

SEQ ID NO: 12 - DNA, 20 bp, Artificial Sequence
  lysA-RA-R2
gaagcctccagcacacgacc

SEQ ID NO: 13 - DNA, 20 bp, Artificial Sequence
  lysA-LA2-R2
tctagctcaggtacacccgt

SEQ ID NO: 14 - DNA, 30 bp, Artificial Sequence
  lysA-RA2-F1
ctgagctagaatttctccccatgacaccag

SEQ ID NO: 15 - DNA, 20 bp, Artificial Sequence
  lysA-LA3-R2
tctagcacaggtacacccgt

SEQ ID NO: 16 - DNA, 30 bp, Artificial Sequence
  lysA-RA3-F1
ctgtgctagaatttctccccatgacaccag